European Patent Application EP 4 667 583 A2, published December 24, 2025. Title: MULTIPLE TAGGING OF INDIVIDUAL LONG DNA FRAGMENTS. Applicant: COMPLETE GENOMICS, INC. Application EP, filed March 17, 2014. The sequence listing filed with the application follows.

SEQUENCE LISTING (2 sequences)

SEQ ID NO: 1 - DNA, 20 bp, synthetic construct
  source 1..20: mol_type = other DNA
ccgcagtagcttacgaatcg

SEQ ID NO: 2 - DNA, 20 bp, synthetic construct
  source 1..20: mol_type = other DNA
gatttaactgagcacttggc